European Patent Specification EP 3 540 057 B1, published September 2, 2026. Title: Malaria Vaccine. Applicant: Sumitomo Dainippon Pharma Co., Ltd. NATIONAL UNIVERSITY CORPORATION EHIME UNIVERSITY. The sequence listing filed with the application follows.

SEQUENCE LISTING (10 sequences)

SEQ ID NO: 1 - DNA, 3261 bp, Plasmodium falciparum
atgttcagaattttttttacccttcttataataatattaatcaagaaaacatcggcaattgatttaatagaaggaattttttatgaaaaaaatgaaatagataaattaacattttctctcgatcatagagttagagataatttaaaaacagatttgattttaaataataatggggaaaatgattatgcttatttaaacaaatacgtttatactatattaaatcgtgattcaacagaaaaaattaaaacatttttttctcataataaagacatgaaatcatgtgattattttatatcaaaagaatataattcaagtgataaaacaaatcaaatatgttataaaaaaacattttgcggagtagtaataccaaatagtgaagaaataaaaacaaataaaataacaaatgacaaactttattgtgcacatttcaattctacacatataatcatttattacatatcacaaccacttttattagaacctcatgttgtttatgaagaaacattttttgaaaaaggaaaaaatgatcaaattaattgccaaggtatgtatatatctctaagatctgtacatgtacatacacacaatgctatattacaacaagaaacacttacatatattaaaaatttatgtgacggaaaaaacaattgtaaattcgattttgattcaataaaatatgaaaataaatcacttactcattatttgttttttattaatatacaatatcaatgcataagtcctctgaatctacaggaaaatgaaatgtgtgacgtatataatgatgatacacataaagcaacatgcaaatatggttttaataaaatagaattattaaaaaatgtttgtgaagaaaattatagatgtacacaagatatatgttcagtaaatcaattttgtgacggagaaaatgaaacatgtacatgcaaaacatcattattaccatcagctaaaaacaattgtgaatacaacgatttatgtacagttttaaattgtcctgaaaattccacatgtgaacaaataggaaatgggaaaaaagctgaatgtaaatgtgaaaatggtaaatattatcacaataataaatgttatacaaaaaatgatttagaattagccataaaaatagaaccacataaaaaagaaaaattttataaaaataatttatatcaaggaaaagcattaaaaccagaatatatttttatgcaatgtgaaaatgggttctctatagaagttattaatgcatatgtatcatgttatagagtttcattcaatctaaacaaattgaaatatgttacagaatcattaaaaaaaatgtgtgatgggaaaaccaaatgtgcttatggaaatacaatagatccaatagatgatttaaatcatcataatatatgtaataattttaatacaatatttaaatatgattatttatgtgtattcaataatcaaaatattacttcagataagaattcacatcttcattctaatataccatcattatataattcaagtattctaccagatattaataaatctaaattccatttgatttcaagaaatagtcgaaccaaccaatatcctcataacaatatatccatgctagaaatacaaaatgaaatatcctcacacaattcaaatcagtttagtacagatccacacacaaatagtaataatataaacaatatgaatattaaaaaggtagaaatcttcagaagtcgtttttcaagtaaattacaatgtcaagggggaaaaataaatattgataaagcaattttaaaaggtggggaaggatgtaatgatttgcttttgacgaattctttaaaatcatattgtaatgatttatcagaatgtgatattggtttaatataccattttgatacttattgtattaatgatcaatatctttttgtatcttacagctgctccaatttatgtaataaatgtcataacaattctacatgctatgggaacagatttaattatgattgtttttgtgataatccttatatttcaaaatatggaaataaattatgtgaacgtccaaatgattgtgaatctgttttgtgttcacaaaatcaagtttgtcaaattcttccaaatgataaattaatatgtcaatgtgaagaaggatataaaaatgttaaaggtaaatgtgttccagacaacaaatgtgatctttcatgcccatcaaacaaagtttgtgttatcgaaaatggaaaacaaacatgtaaatgttcagaacgttttgttctagagaatggtgtgtgtatatgtgctaatgattataaaatggaagatggtattaattgtatagccaaaaataaatgtaaaagaaaagaatatgaaaatatttgtacaaatccaaatgaaatgtgtgcttataatgaagaaacagatattgtaaaatgtgaatgtaaagaacattattatagatcatcaagaggtgaatgtatattaaatgattattgtaaagatattaattgtaaagaaaatgaagaatgttctattgtaaactttaaaccagaatgtgtatgtaaagaaaatcttaaaaaaaataataaaggagaatgtatttatgaaaactcctgtttaattaatgaagggaattgtccaaaagattcaaaatgtatttatagagaatataaaccacatgaatgtgtatgtaataaacaaggtcatgtagctgtcaatggaaaatgtgttttagaagataaatgtgtacataataaaaaatgttcagaaaattctatatgtgtaaatgtaatgaataaagaaccaatatgtgtatgtacatataattattataaaaaagatggtgtatgtttaatacaaaacccttgtctaaaagataatggaggctgctctagaaattcagagtgtacatttaaatatagtaaaattaattgtacatgtaaagaaaattataaaaataaagatgattcttgtgtacctaatacaaatgagtatgatgaaagttttacattccaatataatgacgatgcatctattattcttggagcatgtggtatgatcgaattttcatatatatataaccaaattatttggaaaataaataactcaaaagaatcttacgtattttattatgattatccaacagcaggtaatatagaagttcaaattaaaaatgaaatatttcacactattatatatttgaaaaaaaaaataggcaatagtgttatctatgatgatttccaagtagatcatcaaacatgtatatatgaaaatgtattttattatagtaatcagaattag

SEQ ID NO: 2 - protein, 1086 aa, Plasmodium falciparum
MFRIFFTLLIIILIKKTSAIDLIEGIFYEKNEIDKLTFSLDHRVRDNLKTDLILNNNGENDYAYLNKYVYTILNRDSTEKIKTFFSHNKDMKSCDYFISKEYNSSDKTNQICYKKTFCGVVIPNSEEIKTNKITNDKLYCAHFNSTHIIIYYISQPLLLEPHVVYEETFFEKGKNDQINCQGMYISLRSVHVHTHNAILQQETLTYIKNLCDGKNNCKFDFDSIKYENKSLTHYLFFINIQYQCISPLNLQENEMCDVYNDDTHKATCKYGFNKIELLKNVCEENYRCTQDICSVNQFCDGENETCTCKTSLLPSAKNNCEYNDLCTVLNCPENSTCEQIGNGKKAECKCENGKYYHNNKCYTKNDLELAIKIEPHKKEKFYKNNLYQGKALKPEYIFMQCENGFSIEVINAYVSCYRVSFNLNKLKYVTESLKKMCDGKTKCAYGNTIDPIDDLNHHNICNNFNTIFKYDYLCVFNNQNITSDKNSHLHSNIPSLYNSSILPDINKSKFHLISRNSRTNQYPHNNISMLEIQNEISSHNSNQFSTDPHTNSNNINNMNIKKVEIFRSRFSSKLQCQGGKINIDKAILKGGEGCNDLLLTNSLKSYCNDLSECDIGLIYHFDTYCINDQYLFVSYSCSNLCNKCHNNSTCYGNRFNYDCFCDNPYISKYGNKLCERPNDCESVLCSQNQVCQILPNDKLICQCEEGYKNVKGKCVPDNKCDLSCPSNKVCVIENGKQTCKCSERFVLENGVCICANDYKMEDGINCIAKNKCKRKEYENICTNPNEMCAYNEETDIVKCECKEHYYRSSRGECILNDYCKDINCKENEECSIVNFKPECVCKENLKKNNKGECIYENSCLINEGNCPKDSKCIYREYKPHECVCNKQGHVAVNGKCVLEDKCVHNKKCSENSICVNVMNKEPICVCTYNYYKKDGVCLIQNPCLKDNGGCSRNSECTFKYSKINCTCKENYKNKDDSCVPNTNEYDESFTFQYNDDASIILGACGMIEFSYIYNQIIWKINNSKESYVFYYDYPTAGNIEVQIKNEIFHTIIYLKKKIGNSVIYDDFQVDHQTCIYENVFYYSNQN

SEQ ID NO: 3 - DNA, 645 bp, Artificial Sequence
  Nucleotide sequence encoding the amino acid sequence at positions 720-934 of SEQ ID NO: 2
tgtgatctttcatgcccatcaaacaaagtttgtgttatcgaaaatggaaaacaaacatgtaaatgttcagaacgttttgttctagagaatggtgtgtgtatatgtgctaatgattataaaatggaagatggtattaattgtatagccaaaaataaatgtaaaagaaaagaatatgaaaatatttgtacaaatccaaatgaaatgtgtgcttataatgaagaaacagatattgtaaaatgtgaatgtaaagaacattattatagatcatcaagaggtgaatgtatattaaatgattattgtaaagatattaattgtaaagaaaatgaagaatgttctattgtaaactttaaaccagaatgtgtatgtaaagaaaatcttaaaaaaaataataaaggagaatgtatttatgaaaactcctgtttaattaatgaagggaattgtccaaaagattcaaaatgtatttatagagaatataaaccacatgaatgtgtatgtaataaacaaggtcatgtagctgtcaatggaaaatgtgttttagaagataaatgtgtacataataaaaaatgttcagaaaattctatatgtgtaaatgtaatgaataaagaaccaatatgtgtatgtacatataattattataaaaaagat

SEQ ID NO: 4 - protein, 215 aa, Artificial Sequence
  Amino acid sequence at positions 720-934 of SEQ ID NO: 2
CDLSCPSNKVCVIENGKQTCKCSERFVLENGVCICANDYKMEDGINCIAKNKCKRKEYENICTNPNEMCAYNEETDIVKCECKEHYYRSSRGECILNDYCKDINCKENEECSIVNFKPECVCKENLKKNNKGECIYENSCLINEGNCPKDSKCIYREYKPHECVCNKQGHVAVNGKCVLEDKCVHNKKCSENSICVNVMNKEPICVCTYNYYKKD

SEQ ID NO: 5 - DNA, 3198 bp, Artificial Sequence
  Wheat codon-optimized sequence encoding the amino acid sequence at positions 21-1086 of SEQ ID NO: 2
gatctgatcgagggcatcttctacgagaagaacgagatcgacaagctcaccttctccctggaccacagggtccgcgataacctcaagacggacctcatcctgaacaacaacggcgagaacgattacgcgtacctgaacaagtatgtgtacaccatcctcaacagggactcaaccgagaagatcaagacgttcttctctcacaacaaggatatgaagtcttgcgactacttcatctccaaggagtacaactccagcgataagaccaaccaaatctgctacaagaagacgttctgcggcgtggtcatcccaaactccgaggagatcaagaccaacaagatcacgaacgacaagctctactgcgcccatttcaactccacccacatcatcatctactacatcagccagccactcctgctggagccgcacgttgtgtacgaggagaccttcttcgagaagggcaagaacgaccaaatcaactgccaggggatgtacatctcactgcggtctgtccacgttcatacccacaacgcgatcctccaacaggagaccctgacgtacatcaagaacctctgcgacggcaagaacaactgcaagttcgacttcgatagcatcaagtacgagaacaagtcgctcacccactacctgttcttcatcaacatccagtaccagtgcatctccccgctcaacctgcaagagaacgagatgtgcgacgtctacaacgacgatacccacaaggccacgtgcaagtacggcttcaacaagatcgagctgctcaagaacgtctgcgaggagaactaccgctgcacccaagatatctgctccgttaaccagttctgcgacggcgagaacgagacctgcacgtgcaagacgtcgctgctcccctcagcgaagaacaactgcgagtacaacgacctctgcaccgtgctgaactgccctgagaacagcacgtgcgagcagatcggcaacgggaagaaggctgagtgcaagtgcgagaacggcaagtactaccataacaacaagtgctacaccaagaacgacctggagctggcgatcaagatcgagccacacaagaaggagaagttctacaagaacaacctctaccaaggcaaggctctgaagccggagtacatcttcatgcagtgcgagaacgggttcagcatcgaggtcatcaacgcctacgtctcgtgctaccgcgtttcattcaacctcaacaagctgaagtatgtgaccgagtccctgaagaagatgtgcgatggcaagaccaagtgcgcgtacgggaacacgatcgacccaatcgacgatctcaaccaccataacatctgcaacaacttcaacaccatcttcaagtacgattacctgtgcgtgttcaacaaccaaaacatcacgtctgacaagaactcccatctccacagcaacatcccctcgctctacaactcgtcaatcctgcctgacatcaacaagtcgaagttccatctgatctccaggaacagccgcaccaaccagtacccacacaacaacatctccatgctggagatccaaaacgagatctcttcccataactcaaaccagttctctaccgacccgcacacgaacagcaacaacatcaacaacatgaacatcaagaaggtcgagatcttccggtcgagattcagctcgaagctgcaatgccagggcgggaagatcaacatcgataaggctatcctcaagggcggggagggctgcaacgacctgctcctgaccaactcgctcaagtcatactgcaacgatctgagcgagtgcgacatcgggctcatctaccatttcgatacctactgcatcaacgaccaatacctgttcgtgtcctacagctgctcgaacctctgcaacaagtgccacaacaactccacctgctacggcaacaggttcaactacgactgcttctgcgataacccatacatcagcaagtacgggaacaagctgtgcgagcgcccgaacgattgcgagtccgtgctctgcagccaaaaccaggtctgccaaatcctcccaaacgacaagctgatctgccagtgcgaggaaggctacaagaacgtgaaggggaagtgcgtcccagacaacaagtgcgatctgtcttgcccgtccaacaaggtgtgcgtcatcgagaacggcaagcagacctgcaagtgcagcgagcggttcgttctggagaacggcgtgtgcatctgcgctaacgattacaagatggaggacgggatcaactgcatcgccaagaacaagtgcaagagaaaggagtacgagaacatctgcaccaaccccaacgagatgtgcgcttacaacgaggagacggacatcgtcaagtgcgagtgcaaggagcactactaccggtcatctagaggcgagtgcatcctcaacgactactgcaaggatatcaactgcaaggagaacgaggagtgctccatcgttaacttcaagcctgagtgcgtgtgcaaggagaacctgaagaagaacaacaagggcgagtgcatctacgagaactcttgcctcatcaacgaggggaactgccccaaggactccaagtgcatctacagggagtacaagcctcatgagtgcgtgtgcaacaagcaaggccacgttgccgtgaacgggaagtgcgtcctggaggacaagtgcgttcacaacaagaagtgcagcgagaactcgatctgcgtcaacgttatgaacaaggagcccatctgcgtgtgcacctacaactactacaagaaggatggcgtctgcctcatccagaacccttgcctgaaggacaacggcgggtgctcacgcaactctgagtgcaccttcaagtactcaaagatcaactgcacgtgcaaggagaactacaagaacaaggacgattcttgcgtgcccaacaccaacgagtacgacgagtcgttcacgttccaatacaacgacgatgcctcaatcatcctcggcgcgtgcgggatgatcgagttctcctacatctacaaccagatcatctggaagatcaacaactccaaggagagctacgttttctactacgactacccgaccgccggcaacatcgaggtgcaaatcaagaacgagatcttccataccatcatctacctcaagaagaagatcgggaactcagtcatctacgacgatttccaagttgaccaccagacctgcatctacgagaacgtgttctactactccaaccagaac

SEQ ID NO: 6 - DNA, 645 bp, Artificial Sequence
  Wheat codon-optimized sequence encoding the amino acid sequence at positions 720-934 of SEQ ID NO: 2
tgcgatctgtcttgcccgtccaacaaggtgtgcgtcatcgagaacggcaagcagacctgcaagtgcagcgagcggttcgttctggagaacggcgtgtgcatctgcgctaacgattacaagatggaggacgggatcaactgcatcgccaagaacaagtgcaagagaaaggagtacgagaacatctgcaccaaccccaacgagatgtgcgcttacaacgaggagacggacatcgtcaagtgcgagtgcaaggagcactactaccggtcatctagaggcgagtgcatcctcaacgactactgcaaggatatcaactgcaaggagaacgaggagtgctccatcgttaacttcaagcctgagtgcgtgtgcaaggagaacctgaagaagaacaacaagggcgagtgcatctacgagaactcttgcctcatcaacgaggggaactgccccaaggactccaagtgcatctacagggagtacaagcctcatgagtgcgtgtgcaacaagcaaggccacgttgccgtgaacgggaagtgcgtcctggaggacaagtgcgttcacaacaagaagtgcagcgagaactcgatctgcgtcaacgttatgaacaaggagcccatctgcgtgtgcacctacaactactacaagaaggat

SEQ ID NO: 7 - DNA, 549 bp, Artificial Sequence
  Nucleotide sequence encoding the amino acid sequence at positions 648-830 of SEQ ID NO: 2
tctacatgctatgggaacagatttaattatgattgtttttgtgataatccttatatttcaaaatatggaaataaattatgtgaacgtccaaatgattgtgaatctgttttgtgttcacaaaatcaagtttgtcaaattcttccaaatgataaattaatatgtcaatgtgaagaaggatataaaaatgttaaaggtaaatgtgttccagacaacaaatgtgatctttcatgcccatcaaacaaagtttgtgttatcgaaaatggaaaacaaacatgtaaatgttcagaacgttttgttctagagaatggtgtgtgtatatgtgctaatgattataaaatggaagatggtattaattgtatagccaaaaataaatgtaaaagaaaagaatatgaaaatatttgtacaaatccaaatgaaatgtgtgcttataatgaagaaacagatattgtaaaatgtgaatgtaaagaacattattatagatcatcaagaggtgaatgtatattaaatgattattgtaaagatattaattgtaaagaaaatgaagaatgt

SEQ ID NO: 8 - protein, 183 aa, Artificial Sequence
  Amino acid sequence at positions 648-830 of SEQ ID NO: 2
STCYGNRFNYDCFCDNPYISKYGNKLCERPNDCESVLCSQNQVCQILPNDKLICQCEEGYKNVKGKCVPDNKCDLSCPSNKVCVIENGKQTCKCSERFVLENGVCICANDYKMEDGINCIAKNKCKRKEYENICTNPNEMCAYNEETDIVKCECKEHYYRSSRGECILNDYCKDINCKENEEC

SEQ ID NO: 9 - DNA, 549 bp, Artificial Sequence
  Wheat codon-optimized sequence encoding the amino acid sequence at positions 648-830 of SEQ ID NO: 2
tccacctgctacggcaacaggttcaactacgactgcttctgcgataacccatacatcagcaagtacgggaacaagctgtgcgagcgcccgaacgattgcgagtccgtgctctgcagccaaaaccaggtctgccaaatcctcccaaacgacaagctgatctgccagtgcgaggaaggctacaagaacgtgaaggggaagtgcgtcccagacaacaagtgcgatctgtcttgcccgtccaacaaggtgtgcgtcatcgagaacggcaagcagacctgcaagtgcagcgagcggttcgttctggagaacggcgtgtgcatctgcgctaacgattacaagatggaggacgggatcaactgcatcgccaagaacaagtgcaagagaaaggagtacgagaacatctgcaccaaccccaacgagatgtgcgcttacaacgaggagacggacatcgtcaagtgcgagtgcaaggagcactactaccggtcatctagaggcgagtgcatcctcaacgactactgcaaggatatcaactgcaaggagaacgaggagtgc

SEQ ID NO: 10 - DNA, 645 bp, Artificial Sequence
  Baculovirus codon-optimized sequence encoding the amino acid sequence at positions 720-934 of SEQ ID NO: 2
tgcgacttgtcttgtccctcaaacaaggtgtgcgtcatcgagaacggaaagcagacctgcaaatgttccgagaggttcgtgctggaaaacggagtctgcatttgtgcaaacgactacaagatggaggatggtatcaactgcattgccaagaacaagtgtaagagaaaagagtacgaaaacatctgcaccaacccaaacgaaatgtgcgcttacaacgaggaaactgatattgtgaagtgcgagtgtaaagaacattactaccgctccagccgtggcgagtgcatcctcaacgactactgcaaggatattaactgtaaagaaaacgaggaatgctctatcgtcaacttcaagccggagtgcgtttgtaaggaaaacctgaagaaaaacaacaagggcgagtgcatctacgaaaactcctgtctcattaacgagggaaactgccctaaggacagcaaatgtatctaccgcgagtacaagccccacgaatgcgtctgtaacaagcaaggtcatgttgctgtgaacggcaagtgcgttctggaggataaatgtgtgcacaacaagaaatgcagtgaaaactcgatctgtgtcaacgttatgaacaaggagcccatctgtgtctgcacctacaactactacaaaaaggac